European Patent Application EP 4 613 770 A1, published September 10, 2025. Title: CD22에 결합하는 항체, 이를 포함하는 이중특이적 항체, 키메라 항원 수용체, 항체 약물 복합체 및 이의 용도. Applicant: 재단법인 아산사회복지재단. The sequence listing filed with the application follows.

SEQUENCE LISTING (59 sequences)

SEQ ID NO: 1 - protein, 8 aa, synthetic construct
SGGSGGYG

SEQ ID NO: 2 - protein, 8 aa, synthetic construct
SGSNNTYG

SEQ ID NO: 3 - protein, 7 aa, synthetic construct
DNDQRPS

SEQ ID NO: 4 - protein, 7 aa, synthetic construct
DNTNRPS

SEQ ID NO: 5 - protein, 10 aa, synthetic construct
GSYDSSYVGI

SEQ ID NO: 6 - protein, 10 aa, synthetic construct
GSRDSTYVGI

SEQ ID NO: 7 - protein, 10 aa, synthetic construct
GFTFSNYCMQ

SEQ ID NO: 8 - protein, 10 aa, synthetic construct
GFTFSNYCMS

SEQ ID NO: 9 - protein, 10 aa, synthetic construct
GFTFSKHGHY

SEQ ID NO: 10 - protein, 10 aa, synthetic construct
GFTFSRHGMY

SEQ ID NO: 11 - protein, 10 aa, synthetic construct
GFSFSDYGMG

SEQ ID NO: 12 - protein, 10 aa, synthetic construct
GFAFGRSSMG

SEQ ID NO: 13 - protein, 17 aa, synthetic construct
GIGSSGTGTYYGSAVRG

SEQ ID NO: 14 - protein, 17 aa, synthetic construct
SISNTGSYTDYGAAVKG

SEQ ID NO: 15 - protein, 17 aa, synthetic construct
FLGSSSSYTDYGAAVKG

SEQ ID NO: 16 - protein, 19 aa, synthetic construct
DYGSDSGCGWGIYAGEIDA

SEQ ID NO: 17 - protein, 19 aa, synthetic construct
DYGSDSGIGWGIYAGEIDA

SEQ ID NO: 18 - protein, 19 aa, synthetic construct
DYGSDSGVGWGIYAGEIDA

SEQ ID NO: 19 - protein, 14 aa, synthetic construct
SAYGGSYGSSSIDA

SEQ ID NO: 20 - protein, 102 aa, synthetic construct
LTQPSSVSANPGETVKITCSGGSGGYGWYQQKSPGSAPVSLIYDNDQRPSDIPSRFSGSKSGSTGTLTITGVQADDEAVYYCGSYDSSYVGIFGAGTTLTVL

SEQ ID NO: 21 - protein, 101 aa, synthetic construct
LTQPPSVSVSPGQTARITCSGGSGGYGWYQQKPGSAPVSVIYDNDQRPSGIPERFSGSSSGTTVTLTISGVQAEDEADYYCGSYDSSYVGIFGGGTKLTVL

SEQ ID NO: 22 - protein, 102 aa, synthetic construct
LTQPSSVSANPGETVKITCSGSNNTYGWYQQKAPGSAPVTVIYDNTNRPSDIPSRFSGSKSGSTNTLTITGVQAEDEAVYFCGSRDSTYVGIFGAGTTLTVL

SEQ ID NO: 23 - protein, 128 aa, synthetic construct
AVTLDESGGGLQTPGGALSLVCKASGFTFSNYCMQWVRQAPGKGLEWVAGIGSSGTGTYYGSAVRGRATISRDNGQSTVRLQLNNLRAEDTGTYYCARDYGSDSGCGWGIYAGEIDAWGHGTEVIVSS

SEQ ID NO: 24 - protein, 128 aa, synthetic construct
EVQLLESGGGLVQPGGSLRLSCAASGFTFSNYCMSWVRQAPGKGLEWVSGIGSSGTGTYYGSAVRGRFTISRDNSKNTLYLQMNSLRAEDTAVYYCARDYGSDSGCGWGIYAGEIDAWGQGTLVTVSS

SEQ ID NO: 25 - protein, 128 aa, synthetic construct
EVQLLESGGGLVQPGGSLRLSCAASGFTFSKHGHYWVRQAPGKGLEWVSGIGSSGTGTYYGSAVRGRFTISRDNSKNTLYLQMNSLRAEDTAVYYCARDYGSDSGIGWGIYAGEIDAWGQGTLVTVSS

SEQ ID NO: 26 - protein, 128 aa, synthetic construct
EVQLLESGGGLVQPGGSLRLSCAASGFTFSRHGMYWVRQAPGKGLEWVSGIGSSGTGTYYGSAVRGRFTISRDNSKNTLYLQMNSLRAEDTAVYYCARDYGSDSGVGWGIYAGEIDAWGQGTLVTVSS

SEQ ID NO: 27 - protein, 123 aa, synthetic construct
AVTLDESGGGLQTPGGGLSLVCKASGFSFSDYGMGWVRQAPGKGLEFVASISNTGSYTDYGAAVKGRATISRDNGQSTLRLQLNNLRAEDTGTYFCAKSAYGGSYGSSSIDAWGHGTEVIVSS

SEQ ID NO: 28 - protein, 123 aa, synthetic construct
AVTLDESGGGLQTPGGGLSLVCKASGFAFGRSSMGWVRQAPGKGLEFVASISNTGSYTDYGAAVKGRATISRDNGQSTLRLQLNNLRAEDTGTYFCAKSAYGGSYGSSSIDAWGHGTEVIVSS

SEQ ID NO: 29 - protein, 123 aa, synthetic construct
AVTLDESGGGLQTPGGGLSLVCKASGFSFSDYGMGWVRQAPGKGLEFVAFLGSSSSYTDYGAAVKGRATISRDNGQSTLRLQLNNLRAEDTGTYFCAKSAYGGSYGSSSIDAWGHGTEVIVSS

SEQ ID NO: 30 - protein, 375 aa, synthetic construct
LTQPSSVSANPGETVKITCSGSNNTYGWYQQKAPGSAPVTVIYDNTNRPSDIPSRFSGSKSGSTNTLTITGVQAEDEAVYFCGSRDSTYVGIFGAGTTLTVLGGGGSGGGGSGGGGSAVTLDESGGGLQTPGGGLSLVCKASGFSFSDYGMGWVRQAPGKGLEFVASISNTGSYTDYGAAVKGRATISRDNGQSTLRLQLNNLRAEDTGTYFCAKSAYGGSYGSSSIDAWGHGTEVIVSSGGGGSGGGGSGGGGSRTVAAPSVFIFPPSDEQLKSGTASVVCLLNNFYPREAKVQWKVDNALQSGNSQESVTEQDSKDSTYSLSSTLTLSKADYEKHKVYACEVTHQGLSSPVTKSFNRGESGGAYPYDVPDYAS

SEQ ID NO: 31 - protein, 380 aa, synthetic construct
LTQPSSVSANPGETVKITCSGGSGGYGWYQQKSPGSAPVSLIYDNDQRPSDIPSRFSGSKSGSTGTLTITGVQADDEAVYYCGSYDSSYVGIFGAGTTLTVLGGGGSGGGGSGGGGSAVTLDESGGGLQTPGGALSLVCKASGFTFSNYCMQWVRQAPGKGLEWVAGIGSSGTGTYYGSAVRGRATISRDNGQSTVRLQLNNLRAEDTGTYYCARDYGSDSGCGWGIYAGEIDAWGHGTEVIVSSGGGGSGGGGSGGGGSRTVAAPSVFIFPPSDEQLKSGTASVVCLLNNFYPREAKVQWKVDNALQSGNSQESVTEQDSKDSTYSLSSTLTLSKADYEKHKVYACEVTHQGLSSPVTKSFNRGESGGAYPYDVPDYAS

SEQ ID NO: 32 - protein, 209 aa, synthetic construct
LTQPSSVSANPGETVKITCSGSNNTYGWYQQKAPGSAPVTVIYDNTNRPSDIPSRFSGSKSGSTNTLTITGVQAEDEAVYFCGSRDSTYVGIFGAGTTLTVLRTVAAPSVFIFPPSDEQLKSGTASVVCLLNNFYPREAKVQWKVDNALQSGNSQESVTEQDSKDSTYSLSSTLTLSKADYEKHKVYACEVTHQGLSSPVTKSFNRGEC

SEQ ID NO: 33 - protein, 450 aa, synthetic construct
AVTLDESGGGLQTPGGGLSLVCKASGFSFSDYGMGWVRQAPGKGLEFVASISNTGSYTDYGAAVKGRATISRDNGQSTLRLQLNNLRAEDTGTYFCAKSAYGGSYGSSSIDAWGHGTEVIVSSASTKGPSVFPLAPCSRSTSESTAALGCLVKDYFPEPVTVSWNSGALTSGVHTFPAVLQSSGLYSLSSVVTVPSSSLGTKTYTCNVDHKPSNTKVDKRVESKYGPPCPPCPAPEFLGGPSVFLFPPKPKDTLMISRTPEVTCVVVDVSQEDPEVQFNWYVDGVEVHNAKTKPREEQFNSTYRVVSVLTVLHQDWLNGKEYKCKVSNKGLPSSIEKTISKAKGQPREPQVYTLPPSQEEMTKNQVSLTCLVKGFYPSDIAVEWESNGQPENNYKTTPPVLDSDGSFFLYSRLTVDKSRWQEGNVFSCSVMHEALHNHYTQKSLSLSLGK

SEQ ID NO: 34 - protein, 209 aa, synthetic construct; identical to SEQ ID NO: 32

SEQ ID NO: 35 - protein, 450 aa, synthetic construct
AVTLDESGGGLQTPGGGLSLVCKASGFAFGRSSMGWVRQAPGKGLEFVASISNTGSYTDYGAAVKGRATISRDNGQSTLRLQLNNLRAEDTGTYFCAKSAYGGSYGSSSIDAWGHGTEVIVSSASTKGPSVFPLAPCSRSTSESTAALGCLVKDYFPEPVTVSWNSGALTSGVHTFPAVLQSSGLYSLSSVVTVPSSSLGTKTYTCNVDHKPSNTKVDKRVESKYGPPCPPCPAPEFLGGPSVFLFPPKPKDTLMISRTPEVTCVVVDVSQEDPEVQFNWYVDGVEVHNAKTKPREEQFNSTYRVVSVLTVLHQDWLNGKEYKCKVSNKGLPSSIEKTISKAKGQPREPQVYTLPPSQEEMTKNQVSLTCLVKGFYPSDIAVEWESNGQPENNYKTTPPVLDSDGSFFLYSRLTVDKSRWQEGNVFSCSVMHEALHNHYTQKSLSLSLGK

SEQ ID NO: 36 - protein, 209 aa, synthetic construct; identical to SEQ ID NO: 32

SEQ ID NO: 37 - protein, 450 aa, synthetic construct
AVTLDESGGGLQTPGGGLSLVCKASGFSFSDYGMGWVRQAPGKGLEFVAFLGSSSSYTDYGAAVKGRATISRDNGQSTLRLQLNNLRAEDTGTYFCAKSAYGGSYGSSSIDAWGHGTEVIVSSASTKGPSVFPLAPCSRSTSESTAALGCLVKDYFPEPVTVSWNSGALTSGVHTFPAVLQSSGLYSLSSVVTVPSSSLGTKTYTCNVDHKPSNTKVDKRVESKYGPPCPPCPAPEFLGGPSVFLFPPKPKDTLMISRTPEVTCVVVDVSQEDPEVQFNWYVDGVEVHNAKTKPREEQFNSTYRVVSVLTVLHQDWLNGKEYKCKVSNKGLPSSIEKTISKAKGQPREPQVYTLPPSQEEMTKNQVSLTCLVKGFYPSDIAVEWESNGQPENNYKTTPPVLDSDGSFFLYSRLTVDKSRWQEGNVFSCSVMHEALHNHYTQKSLSLSLGK

SEQ ID NO: 38 - protein, 208 aa, synthetic construct
LTQPPSVSVSPGQTARITCSGGSGGYGWYQQKPGSAPVSVIYDNDQRPSGIPERFSGSSSGTTVTLTISGVQAEDEADYYCGSYDSSYVGIFGGGTKLTVLRTVAAPSVFIFPPSDEQLKSGTASVVCLLNNFYPREAKVQWKVDNALQSGNSQESVTEQDSKDSTYSLSSTLTLSKADYEKHKVYACEVTHQGLSSPVTKSFNRGEC

SEQ ID NO: 39 - protein, 455 aa, synthetic construct
EVQLLESGGGLVQPGGSLRLSCAASGFTFSNYCMSWVRQAPGKGLEWVSGIGSSGTGTYYGSAVRGRFTISRDNSKNTLYLQMNSLRAEDTAVYYCARDYGSDSGCGWGIYAGEIDAWGQGTLVTVSSASTKGPSVFPLAPCSRSTSESTAALGCLVKDYFPEPVTVSWNSGALTSGVHTFPAVLQSSGLYSLSSVVTVPSSSLGTKTYTCNVDHKPSNTKVDKRVESKYGPPCPPCPAPEFLGGPSVFLFPPKPKDTLMISRTPEVTCVVVDVSQEDPEVQFNWYVDGVEVHNAKTKPREEQFNSTYRVVSVLTVLHQDWLNGKEYKCKVSNKGLPSSIEKTISKAKGQPREPQVYTLPPSQEEMTKNQVSLTCLVKGFYPSDIAVEWESNGQPENNYKTTPPVLDSDGSFFLYSRLTVDKSRWQEGNVFSCSVMHEALHNHYTQKSLSLSLGK

SEQ ID NO: 40 - protein, 208 aa, synthetic construct; identical to SEQ ID NO: 38

SEQ ID NO: 41 - protein, 455 aa, synthetic construct
EVQLLESGGGLVQPGGSLRLSCAASGFTFSKHGHYWVRQAPGKGLEWVSGIGSSGTGTYYGSAVRGRFTISRDNSKNTLYLQMNSLRAEDTAVYYCARDYGSDSGIGWGIYAGEIDAWGQGTLVTVSSASTKGPSVFPLAPCSRSTSESTAALGCLVKDYFPEPVTVSWNSGALTSGVHTFPAVLQSSGLYSLSSVVTVPSSSLGTKTYTCNVDHKPSNTKVDKRVESKYGPPCPPCPAPEFLGGPSVFLFPPKPKDTLMISRTPEVTCVVVDVSQEDPEVQFNWYVDGVEVHNAKTKPREEQFNSTYRVVSVLTVLHQDWLNGKEYKCKVSNKGLPSSIEKTISKAKGQPREPQVYTLPPSQEEMTKNQVSLTCLVKGFYPSDIAVEWESNGQPENNYKTTPPVLDSDGSFFLYSRLTVDKSRWQEGNVFSCSVMHEALHNHYTQKSLSLSLGK

SEQ ID NO: 42 - protein, 208 aa, synthetic construct; identical to SEQ ID NO: 38

SEQ ID NO: 43 - protein, 455 aa, synthetic construct
EVQLLESGGGLVQPGGSLRLSCAASGFTFSRHGMYWVRQAPGKGLEWVSGIGSSGTGTYYGSAVRGRFTISRDNSKNTLYLQMNSLRAEDTAVYYCARDYGSDSGVGWGIYAGEIDAWGQGTLVTVSSASTKGPSVFPLAPCSRSTSESTAALGCLVKDYFPEPVTVSWNSGALTSGVHTFPAVLQSSGLYSLSSVVTVPSSSLGTKTYTCNVDHKPSNTKVDKRVESKYGPPCPPCPAPEFLGGPSVFLFPPKPKDTLMISRTPEVTCVVVDVSQEDPEVQFNWYVDGVEVHNAKTKPREEQFNSTYRVVSVLTVLHQDWLNGKEYKCKVSNKGLPSSIEKTISKAKGQPREPQVYTLPPSQEEMTKNQVSLTCLVKGFYPSDIAVEWESNGQPENNYKTTPPVLDSDGSFFLYSRLTVDKSRWQEGNVFSCSVMHEALHNHYTQKSLSLSLGK

SEQ ID NO: 44 - protein, 620 aa, synthetic construct
LTQPSSVSANPGETVKITCSGSNNTYGWYQQKAPGSAPVTVIYDNTNRPSDIPSRFSGSKSGSTNTLTITGVQAEDEAVYFCGSRDSTYVGIFGAGTTLTVLGGGGSGGGGSGGGGSAVTLDESGGGLQTPGGGLSLVCKASGFSFSDYGMGWVRQAPGKGLEFVASISNTGSYTDYGAAVKGRATISRDNGQSTLRLQLNNLRAEDTGTYFCAKSAYGGSYGSSSIDAWGHGTEVIVSSGGGGSGGGGSGGGGSRTVAAPSVFIFPPSDEQLKSGTASVVCLLNNFYPREAKVQWKVDNALQSGNSQESVTEQDSKDSTYSLSSTLTLSKADYEKHKVYACEVTHQGLSLPVTKSFNRGESGGGGSGGGGSGGGGSELDLTQTPASVSAAVGGTVTINCQSSQSPYSNEWLSWYQQKPGQAPKVLISRISTLASGVSSRFKGSGSGTQFTLTISDLECGDAATYFCAGGYNFGLFPFGGGTELEILSSGGGGSGGGGGGSSRSSQSVKESEGRLVTPGGSLTLTCTVSGIDLSRDWMNWVRQAPGEGLEWIGAIGRSGDTYYATWAKGRFTISKTSSRTVTLTVTDLQRSDTATYFCARIPYFGWNNGDIWGPGTLVTI

SEQ ID NO: 45 - protein, 625 aa, synthetic construct
LTQPSSVSANPGETVKITCSGGSGGYGWYQQKSPGSAPVSLIYDNDQRPSDIPSRFSGSKSGSTGTLTITGVQADDEAVYYCGSYDSSYVGIFGAGTTLTVLGGGGSGGGGSGGGGSAVTLDESGGGLQTPGGALSLVCKASGFTFSNYCMQWVRQAPGKGLEWVAGIGSSGTGTYYGSAVRGRATISRDNGQSTVRLQLNNLRAEDTGTYYCARDYGSDSGCGWGIYAGEIDAWGHGTEVIVSSGGGGSGGGGSGGGGSRTVAAPSVFIFPPSDEQLKSGTASVVCLLNNFYPREAKVQWKVDNALQSGNSQESVTEQDSKDSTYSLSSTLTLSKADYEKHKVYACEVTHQGLSLPVTKSFNRGESGGGGSGGGGSGGGGSELDLTQTPASVSAAVGGTVTINCQSSQSPYSNEWLSWYQQKPGQAPKVLISRISTLASGVSSRFKGSGSGTQFTLTISDLECGDAATYFCAGGYNFGLFPFGGGTELEILSSGGGGSGGGGGGSSRSSQSVKESEGRLVTPGGSLTLTCTVSGIDLSRDWMNWVRQAPGEGLEWIGAIGRSGDTYYATWAKGRFTISKTSSRTVTLTVTDLQRSDTATYFCARIPYFGWNNGDIWGPGTLVTI

SEQ ID NO: 46 - protein, 625 aa, synthetic construct
DIQMTQSPSSLSASVGDRVTITCRASQDVNTAVAWYQQKPGKAPKLLIYSASFLYSGVPSRFSGSRSGTDFTLTISSLQPEDFATYYCQQHYTTPPTFGQGTKVEIKGGSSRSSSSGGGGSGGGGEVQLVESGGGLVQPGGSLRLSCAASGFNIKDTYIHWVRQAPGKGLEWVARIYPTNGYTRYADSVKGRFTISADTSKNTAYLQMNSLRAEDTAVYYCSRWGGDGFYAMDYWGQGTLVTVSSGGGGSGGGGSGGGGSRTVAAPSVFIFPPSDEQLKSGTASVVCLLNNFYPREAKVQWKVDNALQSGNSQESVTEQDSKDSTYSLSSTLTLSKADYEKHKVYACEVTHQGLSLPVTKSFNRGESGGGGSGGGGSGGGGSELDLTQTPASVSAAVGGTVTINCQSSQSPYSNEWLSWYQQKPGQAPKVLISRISTLASGVSSRFKGSGSGTQFTLTISDLECGDAATYFCAGGYNFGLFPFGGGTELEILSSGGGGSGGGGGGSSRSSQSVKESEGRLVTPGGSLTLTCTVSGIDLSRDWMNWVRQAPGEGLEWIGAIGRSGDTYYATWAKGRFTISKTSSRTVTLTVTDLQRSDTATYFCARIPYFGWNNGDIWGPGTLVTI

SEQ ID NO: 47 - protein, 499 aa, synthetic construct
LTQPSSVSANPGETVKITCSGGSGGYGWYQQKSPGSAPVSLIYDNDQRPSDIPSRFSGSKSGSTGTLTITGVQADDEAVYYCGSYDSSYVGIFGAGTTLTVLGGGGSGGGGSGGGGSAVTLDESGGGLQTPGGALSLVCKASGFTFSNYCMQWVRQAPGKGLEWVAGIGSSGTGTYYGSAVRGRATISRDNGQSTVRLQLNNLRAEDTGTYYCARDYGSDSGCGWGIYAGEIDAWGHGTEVIVSSGGGGSDIKLQQSGAELARPGASVKMSCKTSGYTFTRYTMHWVKQRPGQGLEWIGYINPSRGYTNYNQKFKDKATLTTDKSSSTAYMQLSSLTSEDSAVYYCARYYDDHYCLDYWGQGTTLTVSSVEGGSGGSGGSGGSGGVDDIQLTQSPAIMSASPGEKVTMTCRASSSVSYMNWYQQKSGTSPKRWIYDTSKVASGVPYRFSGSGSGTSYSLTISSMEAEDAATYYCQQWSSNPLTFGAGTKLELKHHHHHH

SEQ ID NO: 48 - protein, 498 aa, synthetic construct
LTQPPSVSVSPGQTARITCSGGSGGYGWYQQKPGSAPVSVIYDNDQRPSGIPERFSGSSSGTTVTLTISGVQAEDEADYYCGSYDSSYVGIFGGGTKLTVLGGGGSGGGGSGGGGSEVQLLESGGGLVQPGGSLRLSCAASGFTFSNYCMSWVRQAPGKGLEWVSGIGSSGTGTYYGSAVRGRFTISRDNSKNTLYLQMNSLRAEDTAVYYCARDYGSDSGCGWGIYAGEIDAWGQGTLVTVSSGGGGSDIKLQQSGAELARPGASVKMSCKTSGYTFTRYTMHWVKQRPGQGLEWIGYINPSRGYTNYNQKFKDKATLTTDKSSSTAYMQLSSLTSEDSAVYYCARYYDDHYCLDYWGQGTTLTVSSVEGGSGGSGGSGGSGGVDDIQLTQSPAIMSASPGEKVTMTCRASSSVSYMNWYQQKSGTSPKRWIYDTSKVASGVPYRFSGSGSGTSYSLTISSMEAEDAATYYCQQWSSNPLTFGAGTKLELKHHHHHH

SEQ ID NO: 49 - protein, 498 aa, synthetic construct
LTQPPSVSVSPGQTARITCSGGSGGYGWYQQKPGSAPVSVIYDNDQRPSGIPERFSGSSSGTTVTLTISGVQAEDEADYYCGSYDSSYVGIFGGGTKLTVLGGGGSGGGGSGGGGSEVQLLESGGGLVQPGGSLRLSCAASGFTFSKHGHYWVRQAPGKGLEWVSGIGSSGTGTYYGSAVRGRFTISRDNSKNTLYLQMNSLRAEDTAVYYCARDYGSDSGIGWGIYAGEIDAWGQGTLVTVSSGGGGSDIKLQQSGAELARPGASVKMSCKTSGYTFTRYTMHWVKQRPGQGLEWIGYINPSRGYTNYNQKFKDKATLTTDKSSSTAYMQLSSLTSEDSAVYYCARYYDDHYCLDYWGQGTTLTVSSVEGGSGGSGGSGGSGGVDDIQLTQSPAIMSASPGEKVTMTCRASSSVSYMNWYQQKSGTSPKRWIYDTSKVASGVPYRFSGSGSGTSYSLTISSMEAEDAATYYCQQWSSNPLTFGAGTKLELKHHHHHH

SEQ ID NO: 50 - protein, 498 aa, synthetic construct
LTQPPSVSVSPGQTARITCSGGSGGYGWYQQKPGSAPVSVIYDNDQRPSGIPERFSGSSSGTTVTLTISGVQAEDEADYYCGSYDSSYVGIFGGGTKLTVLGGGGSGGGGSGGGGSEVQLLESGGGLVQPGGSLRLSCAASGFTFSRHGMYWVRQAPGKGLEWVSGIGSSGTGTYYGSAVRGRFTISRDNSKNTLYLQMNSLRAEDTAVYYCARDYGSDSGVGWGIYAGEIDAWGQGTLVTVSSGGGGSDIKLQQSGAELARPGASVKMSCKTSGYTFTRYTMHWVKQRPGQGLEWIGYINPSRGYTNYNQKFKDKATLTTDKSSSTAYMQLSSLTSEDSAVYYCARYYDDHYCLDYWGQGTTLTVSSVEGGSGGSGGSGGSGGVDDIQLTQSPAIMSASPGEKVTMTCRASSSVSYMNWYQQKSGTSPKRWIYDTSKVASGVPYRFSGSGSGTSYSLTISSMEAEDAATYYCQQWSSNPLTFGAGTKLELKHHHHHH

SEQ ID NO: 51 - protein, 494 aa, synthetic construct
LTQPSSVSANPGETVKITCSGSNNTYGWYQQKAPGSAPVTVIYDNTNRPSDIPSRFSGSKSGSTNTLTITGVQAEDEAVYFCGSRDSTYVGIFGAGTTLTVLGGGGSGGGGSGGGGSAVTLDESGGGLQTPGGGLSLVCKASGFSFSDYGMGWVRQAPGKGLEFVASISNTGSYTDYGAAVKGRATISRDNGQSTLRLQLNNLRAEDTGTYFCAKSAYGGSYGSSSIDAWGHGTEVIVSSGGGGSDIKLQQSGAELARPGASVKMSCKTSGYTFTRYTMHWVKQRPGQGLEWIGYINPSRGYTNYNQKFKDKATLTTDKSSSTAYMQLSSLTSEDSAVYYCARYYDDHYCLDYWGQGTTLTVSSVEGGSGGSGGSGGSGGVDDIQLTQSPAIMSASPGEKVTMTCRASSSVSYMNWYQQKSGTSPKRWIYDTSKVASGVPYRFSGSGSGTSYSLTISSMEAEDAATYYCQQWSSNPLTFGAGTKLELKHHHHHH

SEQ ID NO: 52 - protein, 494 aa, synthetic construct
LTQPSSVSANPGETVKITCSGSNNTYGWYQQKAPGSAPVTVIYDNTNRPSDIPSRFSGSKSGSTNTLTITGVQAEDEAVYFCGSRDSTYVGIFGAGTTLTVLGGGGSGGGGSGGGGSAVTLDESGGGLQTPGGGLSLVCKASGFAFGRSSMGWVRQAPGKGLEFVASISNTGSYTDYGAAVKGRATISRDNGQSTLRLQLNNLRAEDTGTYFCAKSAYGGSYGSSSIDAWGHGTEVIVSSGGGGSDIKLQQSGAELARPGASVKMSCKTSGYTFTRYTMHWVKQRPGQGLEWIGYINPSRGYTNYNQKFKDKATLTTDKSSSTAYMQLSSLTSEDSAVYYCARYYDDHYCLDYWGQGTTLTVSSVEGGSGGSGGSGGSGGVDDIQLTQSPAIMSASPGEKVTMTCRASSSVSYMNWYQQKSGTSPKRWIYDTSKVASGVPYRFSGSGSGTSYSLTISSMEAEDAATYYCQQWSSNPLTFGAGTKLELKHHHHHH

SEQ ID NO: 53 - protein, 378 aa, synthetic construct
LTQPSSVSANPGETVKITCSGSNNTYGWYQQKAPGSAPVTVIYDNTNRPSDIPSRFSGSKSGSTNTLTITGVQAEDEAVYFCGSRDSTYVGIFGAGTTLTVLGGGGSGGGGSGGGGSAVTLDESGGGLQTPGGGLSLVCKASGFSFSDYGMGWVRQAPGKGLEFVAFLGSSSSYTDYGAAVKGRATISRDNGQSTLRLQLNNLRAEDTGTYFCAKSAYGGSYGSSSIDAWGHGTEVIVSSGGGGSDIKLQQSGAELARPGASVKMSCKTSGYTFTRYTMHWVKQRPGQGLEWIGYINPSRGYTNYNQKFKDKATLTTDKSSSTAYMQLSSLTSEDSAVYYCARYYDDHYCLDYWGQGTTLTVSSVEGGSGGSGGSGGS

SEQ ID NO: 54 - protein, 504 aa, synthetic construct
DIQLTQSPASLAVSLGQRATISCKASQSVDYDGDSYLNWYQQIPGQPPKLLIYDASNLVSGIPPRFSGSGSGTDFTLNIHPVEKVDAATYHCQQSTEDPWTFGGGTKLEIKGGGGSGGGGSGGGGSQVQLQQSGAELVRPGSSVKISCKASGYAFSSYWMNWVKQRPGQGLEWIGQIWPGDGDTNYNGKFKGKATLTADESSSTAYMQLSSLASEDSAVYFCARRETTTVGRYYYAMDYWGQGTTVTVSSGGGGSDIKLQQSGAELARPGASVKMSCKTSGYTFTRYTMHWVKQRPGQGLEWIGYINPSRGYTNYNQKFKDKATLTTDKSSSTAYMQLSSLTSEDSAVYYCARYYDDHYCLDYWGQGTTLTVSSVEGGSGGSGGSGGSGGVDDIQLTQSPAIMSASPGEKVTMTCRASSSVSYMNWYQQKSGTSPKRWIYDTSKVASGVPYRFSGSGSGTSYSLTISSMEAEDAATYYCQQWSSNPLTFGAGTKLELKHHHHHH

SEQ ID NO: 55 - protein, 496 aa, synthetic construct
MALPVTALLLPLALLLHAARPEQKLISEEDLDIQMTQTTSSLSASLGDRVTISCRASQDISKYLNWYQQKPDGTVKLLIYHTSRLHSGVPSRFSGSGSGTDYSLTISNLEQEDIATYFCQQGNTLPYTFGGGTKLEITGGGGSGGGGSGGGGSEVKLQESGPGLVAPSQSLSVTCTVSGVSLPDYGVSWIRQPPRKGLEWLGVIWGSETTYYNSALKSRLTIIKDNSKSQVFLKMNSLQTDDTAIYYCAKHYYYGGSYAMDYWGQGTSVTVSSTTTPAPRPPTPAPTIASQPLSLRPEACRPAAGGAVHTRGLDFACDIYIWAPLAGTCGVLLLSLVITLYCKRGRKKLLYIFKQPFMRPVQTTQEEDGCSCRFPEEEEGGCELRVKFSRSADAPAYKQGQNQLYNELNLGRREEYDVLDKRRGRDPEMGGKPRRKNPQEGLYNELQKDKMAEAYSEIGMKGERRRGKGHDGLYQGLSTATKDTYDALHMQALPPR

SEQ ID NO: 56 - protein, 502 aa, synthetic construct
MALPVTALLLPLALLLHAARPEQKLISEEDLLTQPSSVSANPGETVKITCSGGSGGYGWYQQKSPGSAPVSLIYDNDQRPSDIPSRFSGSKSGSTGTLTITGVQADDEAVYYCGSYDSSYVGIFGAGTTLTVLGQSSRSSGGGGSSGGGGSAVTLDESGGGLQTPGGALSLVCKASGFTFSNYCMQWVRQAPGKGLEWVAGIGSSGTGTYYGSAVRGRATISRDNGQSTVRLQLNNLRAEDTGTYYCARDYGSDSGCGWGIYAGEIDAWGHGTEVIVSSTTTPAPRPPTPAPTIASQPLSLRPEACRPAAGGAVHTRGLDFACDIYIWAPLAGTCGVLLLSLVITLYCKRGRKKLLYIFKQPFMRPVQTTQEEDGCSCRFPEEEEGGCELRVKFSRSADAPAYKQGQNQLYNELNLGRREEYDVLDKRRGRDPEMGGKPRRKNPQEGLYNELQKDKMAEAYSEIGMKGERRRGKGHDGLYQGLSTATKDTYDALHMQALPPR

SEQ ID NO: 57 - protein, 768 aa, synthetic construct
MALPVTALLLPLALLLHAARPEQKLISEEDLGRADIQMTQTTSSLSASLGDRVTISCRASQDISKYLNWYQQKPDGTVKLLIYHTSRLHSGVPSRFSGSGSGTDYSLTISNLEQEDIATYFCQQGNTLPYTFGGGTKLEITGSTSGSGKPGSGEGSTKGEVKLQESGPGLVAPSQSLSVTCTVSGVSLPDYGVSWIRQPPRKGLEWLGVIWGSETTYYNSALKSRLTIIKDNSKSQVFLKMNSLQTDDTAIYYCAKHYYYGGSYAMDYWGQGTSVTVSSGGGGSGGGGSGGGGSLTQPSSVSANPGETVKITCSGGSGGYGWYQQKSPGSAPVSLIYDNDQRPSDIPSRFSGSKSGSTGTLTITGVQADDEAVYYCGSYDSSYVGIFGAGTTLTVLGQSSRSSGGGGSSGGGGSAVTLDESGGGLQTPGGALSLVCKASGFTFSNYCMQWVRQAPGKGLEWVAGIGSSGTGTYYGSAVRGRATISRDNGQSTVRLQLNNLRAEDTGTYYCARDYGSDSGCGWGIYAGEIDAWGHGTEVIVSSLINTTTPAPRPPTPAPTIASQPLSLRPEACRPAAGGAVHTRGLDFACDIYIWAPLAGTCGVLLLSLVITLYCKRGRKKLLYIFKQPFMRPVQTTQEEDGCSCRFPEEEEGGCELRVKFSRSADAPAYKQGQNQLYNELNLGRREEYDVLDKRRGRDPEMGGKPRRKNPQEGLYNELQKDKMAEAYSEIGMKGERRRGKGHDGLYQGLSTATKDTYDALHMQALPPR

SEQ ID NO: 58 - protein, 768 aa, synthetic construct
MALPVTALLLPLALLLHAARPEQKLISEEDLGRALTQPSSVSANPGETVKITCSGGSGGYGWYQQKSPGSAPVSLIYDNDQRPSDIPSRFSGSKSGSTGTLTITGVQADDEAVYYCGSYDSSYVGIFGAGTTLTVLGQSSRSSGGGGSSGGGGSAVTLDESGGGLQTPGGALSLVCKASGFTFSNYCMQWVRQAPGKGLEWVAGIGSSGTGTYYGSAVRGRATISRDNGQSTVRLQLNNLRAEDTGTYYCARDYGSDSGCGWGIYAGEIDAWGHGTEVIVSSGGGGSGGGGSGGGGSDIQMTQTTSSLSASLGDRVTISCRASQDISKYLNWYQQKPDGTVKLLIYHTSRLHSGVPSRFSGSGSGTDYSLTISNLEQEDIATYFCQQGNTLPYTFGGGTKLEITGSTSGSGKPGSGEGSTKGEVKLQESGPGLVAPSQSLSVTCTVSGVSLPDYGVSWIRQPPRKGLEWLGVIWGSETTYYNSALKSRLTIIKDNSKSQVFLKMNSLQTDDTAIYYCAKHYYYGGSYAMDYWGQGTSVTVSSLINTTTPAPRPPTPAPTIASQPLSLRPEACRPAAGGAVHTRGLDFACDIYIWAPLAGTCGVLLLSLVITLYCKRGRKKLLYIFKQPFMRPVQTTQEEDGCSCRFPEEEEGGCELRVKFSRSADAPAYKQGQNQLYNELNLGRREEYDVLDKRRGRDPEMGGKPRRKNPQEGLYNELQKDKMAEAYSEIGMKGERRRGKGHDGLYQGLSTATKDTYDALHMQALPPR

SEQ ID NO: 59 - protein, 745 aa, synthetic construct
MALPVTALLLPLALLLHAARPEQKLISEEDLGRADIQMTQTTSSLSASLGDRVTISCRASQDISKYLNWYQQKPDGTVKLLIYHTSRLHSGVPSRFSGSGSGTDYSLTISNLEQEDIATYFCQQGNTLPYTFGGGTKLEITGGGGSAVTLDESGGGLQTPGGALSLVCKASGFTFSNYCMQWVRQAPGKGLEWVAGIGSSGTGTYYGSAVRGRATISRDNGQSTVRLQLNNLRAEDTGTYYCARDYGSDSGCGWGIYAGEIDAWGHGTEVIVSSGSTSGSGKPGSGEGSTKGLTQPSSVSANPGETVKITCSGGSGGYGWYQQKSPGSAPVSLIYDNDQRPSDIPSRFSGSKSGSTGTLTITGVQADDEAVYYCGSYDSSYVGIFGAGTTLTVLGGGGSEVKLQESGPGLVAPSQSLSVTCTVSGVSLPDYGVSWIRQPPRKGLEWLGVIWGSETTYYNSALKSRLTIIKDNSKSQVFLKMNSLQTDDTAIYYCAKHYYYGGSYAMDYWGQGTSVTVSSLINTTTPAPRPPTPAPTIASQPLSLRPEACRPAAGGAVHTRGLDFACDIYIWAPLAGTCGVLLLSLVITLYCKRGRKKLLYIFKQPFMRPVQTTQEEDGCSCRFPEEEEGGCELRVKFSRSADAPAYKQGQNQLYNELNLGRREEYDVLDKRRGRDPEMGGKPRRKNPQEGLYNELQKDKMAEAYSEIGMKGERRRGKGHDGLYQGLSTATKDTYDALHMQALPPR